European Patent Application EP 4 269 579 A2, published November 1, 2023. Title: GENE THERAPY CONSTRUCTS FOR TREATING WILSON DISEASE. Applicant: ULTRAGENYX PHARMACEUTICAL INC. Application EP, filed September 12, 2023. The sequence listing filed with the application follows.

SEQUENCE LISTING (15 sequences)

SEQ ID NO: 1 - DNA, 3603 bp, synthetic construct
  misc_feature 1..3603: note = Description of artificial sequence: Del 1-3 ATP7B, native
  misc_feature 223..225: note = Nucleotides 223-225 encode for serine residue S340 (numbering based on wild-type protein sequence)
  misc_feature 226..228: note = Nucleotides 226-228 encode for serine residue S341 (numbering based on wild-type protein sequence)
  source 1..3603: mol_type = other DNA
atgcctgagcaggagagacagatcacagccagagaaggggccagtcggaaaatcttatctaagctttctttgcctacccgtgcctgggaaccagcaatgaagaagagttttgcttttgacaatgttggctatgaaggtggtctggatggcctgggcccttcttctcaggtggccaccagcacagtcagggatggagccgaagggagtgggacagatcacaggtcttccagttctcattcccctggctccccaccgagaaaccaggtccagggcacatgcagtaccactctgattgccattgccggcatgacctgtgcatcctgtgtccattccattgaaggcatgatctcccaactggaaggggtgcagcaaatatcggtgtctttggccgaagggactgcaacagttctttataatccctctgtaattagcccagaagaactcagagctgctatagaagacatgggatttgaggcttcagtcgtttctgaaagctgttctactaaccctcttggaaaccacagtgctgggaattccatggtgcaaactacagatggtacacctacatctgtgcaggaagtggctccccacactgggaggctccctgcaaaccatgccccggacatcttggcaaagtccccacaatcaaccagagcagtggcaccgcagaagtgcttcttacagatcaaaggcatgacctgtgcatcctgtgtgtctaacatagaaaggaatctgcagaaagaagctggtgttctctccgtgttggttgccttgatggcaggaaaggcagagatcaagtatgacccagaggtcatccagcccctcgagatagctcagttcatccaggacctgggttttgaggcagcagtcatggaggactacgcaggctccgatggcaacattgagctgacaatcacagggatgacctgcgcgtcctgtgtccacaacatagagtccaaactcacgaggacaaatggcatcacttatgcctccgttgcccttgccaccagcaaagcccttgttaagtttgacccggaaattatcggtccacgggatattatcaaaattattgaggaaattggctttcatgcttccctggcccagagaaaccccaacgctcatcacttggaccacaagatggaaataaagcagtggaagaagtctttcctgtgcagcctggtgtttggcatccctgtcatggccttaatgatctatatgctgatacccagcaacgagccccaccagtccatggtcctggaccacaacatcattccaggactgtccattctaaatctcatcttctttatcttgtgtacctttgtccagctcctcggtgggtggtacttctacgttcaggcctacaaatctctgagacacaggtcagccaacatggacgtgctcatcgtcctggccacaagcattgcttatgtttattctctggtcatcctggtggttgctgtggctgagaaggcggagaggagccctgtgacattcttcgacacgccccccatgctctttgtgttcattgccctgggccggtggctggaacacttggcaaagagcaaaacctcagaagccctggctaaactcatgtctctccaagccacagaagccaccgttgtgacccttggtgaggacaatttaatcatcagggaggagcaagtccccatggagctggtgcagcggggcgatatcgtcaaggtggtccctgggggaaagtttccagtggatgggaaagtcctggaaggcaataccatggctgatgagtccctcatcacaggagaagccatgccagtcactaagaaacccggaagcactgtaattgcggggtctataaatgcacatggctctgtgctcattaaagctacccacgtgggcaatgacaccactttggctcagattgtgaaactggtggaagaggctcagatgtcaaaggcacccattcagcagctggctgaccggtttagtggatattttgtcccatttatcatcatcatgtcaactttgacgttggtggtatggattgtaatcggttttatcgattttggtgttgttcagagatactttcctaaccccaacaagcacatctcccagacagaggtgatcatccggtttgctttccagacgtccatcacggtgctgtgcattgcctgcccctgctccctggggctggccacgcccacggctgtcatggtgggcaccggggtggccgcgcagaacggcatcctcatcaagggaggcaagcccctggagatggcgcacaagataaagactgtgatgtttgacaagactggcaccattacccatggcgtccccagggtcatgcgggtgctcctgctgggggatgtggccacactgcccctcaggaaggttctggctgtggtggggactgcggaggccagcagtgaacaccccttgggcgtggcagtcaccaaatactgtaaagaggaacttggaacagagaccttgggatactgcacggacttccaggcagtgccaggctgtggaattgggtgcaaagtcagcaacgtggaaggcatcctggcccacagtgagcgccctttgagtgcaccggccagtcacctgaatgaggctggcagccttcccgcagaaaaagatgcagtcccccagaccttctctgtgctgattggaaaccgtgagtggctgaggcgcaacggtttaaccatttctagcgatgtcagtgacgctatgacagaccacgagatgaaaggacagacagccatcctggtggctattgacggtgtgctctgtgggatgatcgcaatcgcagacgctgtcaagcaggaggctgccctggctgtgcacacgctgcagagcatgggtgtggacgtggttctgatcacgggggacaaccggaagacagccagagctattgccacccaggttggcatcaacaaagtctttgcagaggtgctgccttcgcacaaggtggccaaggtccaggagctccagaataaagggaagaaagtcgccatggtgggggatggggtcaatgactccccggccttggcccaggcagacatgggtgtggccattggcaccggcacggatgtggccatcgaggcagccgacgtcgtccttatcagaaatgatttgctggatgtggtggctagcattcacctttccaagaggactgtccgaaggatacgcatcaacctggtcctggcactgatttataacctggttgggatacccattgcagcaggtgtcttcatgcccatcggcattgtgctgcagccctggatgggctcagcggccatggcagcctcctctgtgtctgtggtgctctcatccctgcagctcaagtgctataagaagcctgacctggagaggtatgaggcacaggcgcatggccacatgaagcccctgacggcatcccaggtcagtgtgcacataggcatggatgacaggtggcgggactcccccagggccacaccatgggaccaggtcagctatgtcagccaggtgtcgctgtcctccctgacgtccgacaagccatctcggcacagcgctgcagcagacgatgatggggacaagtggtctctgctcctgaatggcagggatgaggagcagtacatctga

SEQ ID NO: 2 - DNA, 145 bp, synthetic construct
  misc_feature 1..145: note = Description of artificial sequence: AAV2 ITR
  source 1..145: mol_type = other DNA
ttggccactccctctctgcgcgctcgctcgctcactgaggccgggcgaccaaaggtcgcccgacgcccgggctttgcccgggcggcctcagtgagcgagcgagcgcgcagagagggagtggccaactccatcactaggggttcct

SEQ ID NO: 3 - DNA, 100 bp, synthetic construct
  misc_feature 1..100: note = Description of artificial sequence: enTTR Enhancer sequence
  source 1..100: mol_type = other DNA
ctacctcgtgatcgcccggcccctgttcaaacatgtcctaatactctgtctctgcaagggtcatcagtagttttccatcttactcaacatcctcccagtg

SEQ ID NO: 4 - DNA, 95 bp, synthetic construct
  misc_feature 1..95: note = Description of artificial sequence: SV40 Small T Intron
  source 1..95: mol_type = other DNA
gctctaaggtaaatataaaatttttaagtgtataatgtgttaaactactgattctaattgtttctctcttttagattccaacctttggaactgat

SEQ ID NO: 5 - DNA, 315 bp, synthetic construct
  misc_feature 1..315: note = Description of artificial sequence: rHBB Intron
  source 1..315: mol_type = other DNA
gtgagcgggcgggacggcccttctcctccgggctgtaattagcgcttggtttaatgacggcttgtttcttttctgtggctgcgtgaaagccttgaggggctccgggagggccctttgtgcggggggagcggctcggggctgtccgcggggggacggctgccttcgggggggacggggcagggcggggttcggcttctggcgtgtgaccggcggctcaagagcctctgctaaccatgttcatgccttcttctttttcctacagctcctgggcaacgtgctggttattgtgctgtctcatcattttggcaaagaatt

SEQ ID NO: 6 - DNA, 215 bp, synthetic construct
  misc_feature 1..215: note = Description of artificial sequence: BGH polyadenylation signal sequence
  source 1..215: mol_type = other DNA
gcctcgactgtgccttctagttgccagccatctgttgtttgcccctcccccgtgccttccttgaccctggaaggtgccactcccactgtcctttcctaataaaatgaggaaattgcatcgcattgtctgagtaggtgtcattctattctggggggtggggtggggcaggacagcaagggggaggattgggaagacaatagcaggcatgctgggga

SEQ ID NO: 7 - DNA, 198 bp, synthetic construct
  misc_feature 1..198: note = Description of artificial sequence: SV40 polyadenylation signal sequence
  source 1..198: mol_type = other DNA
gatccagacatgataagatacattgatgagtttggacaaaccacaactagaatgcagtgaaaaaaatgctttatttgtgaaatttgtgatgctattgctttatttgtaaccattataagctgcaataaacaagttaacaacaacaattgcattcattttatgtttcaggttcagggggaggtgtgggaggttttttag

SEQ ID NO: 8 - protein, 1200 aa, synthetic construct
  REGION 1..1200: note = Description of artificial sequence: DEL 1-3 ATP7B Native, protein
  SITE 75: note = MISC_FEATURE - Amino acid residue at position 75 corresponds to Serine S340 (numbering based on wild-type protein sequence)
  SITE 76: note = MISC_FEATURE - Amino acid residue at position 76 corresponds to Serine S341 (numbering based on wild-type protein sequence)
MPEQERQITAREGASRKILSKLSLPTRAWEPAMKKSFAFDNVGYEGGLDGLGPSSQVATSTVRDGAEGSGTDHRSSSSHSPGSPPRNQVQGTCSTTLIAIAGMTCASCVHSIEGMISQLEGVQQISVSLAEGTATVLYNPSVISPEELRAAIEDMGFEASVVSESCSTNPLGNHSAGNSMVQTTDGTPTSVQEVAPHTGRLPANHAPDILAKSPQSTRAVAPQKCFLQIKGMTCASCVSNIERNLQKEAGVLSVLVALMAGKAEIKYDPEVIQPLEIAQFIQDLGFEAAVMEDYAGSDGNIELTITGMTCASCVHNIESKLTRTNGITYASVALATSKALVKFDPEIIGPRDIIKIIEEIGFHASLAQRNPNAHHLDHKMEIKQWKKSFLCSLVFGIPVMALMIYMLIPSNEPHQSMVLDHNIIPGLSILNLIFFILCTFVQLLGGWYFYVQAYKSLRHRSANMDVLIVLATSIAYVYSLVILVVAVAEKAERSPVTFFDTPPMLFVFIALGRWLEHLAKSKTSEALAKLMSLQATEATVVTLGEDNLIIREEQVPMELVQRGDIVKVVPGGKFPVDGKVLEGNTMADESLITGEAMPVTKKPGSTVIAGSINAHGSVLIKATHVGNDTTLAQIVKLVEEAQMSKAPIQQLADRFSGYFVPFIIIMSTLTLVVWIVIGFIDFGVVQRYFPNPNKHISQTEVIIRFAFQTSITVLCIACPCSLGLATPTAVMVGTGVAAQNGILIKGGKPLEMAHKIKTVMFDKTGTITHGVPRVMRVLLLGDVATLPLRKVLAVVGTAEASSEHPLGVAVTKYCKEELGTETLGYCTDFQAVPGCGIGCKVSNVEGILAHSERPLSAPASHLNEAGSLPAEKDAVPQTFSVLIGNREWLRRNGLTISSDVSDAMTDHEMKGQTAILVAIDGVLCGMIAIADAVKQEAALAVHTLQSMGVDVVLITGDNRKTARAIATQVGINKVFAEVLPSHKVAKVQELQNKGKKVAMVGDGVNDSPALAQADMGVAIGTGTDVAIEAADVVLIRNDLLDVVASIHLSKRTVRRIRINLVLALIYNLVGIPIAAGVFMPIGIVLQPWMGSAAMAASSVSVVLSSLQLKCYKKPDLERYEAQAHGHMKPLTASQVSVHIGMDDRWRDSPRATPWDQVSYVSQVSLSSLTSDKPSRHSAAADDDGDKWSLLLNGRDEEQYI

SEQ ID NO: 9 - DNA, 2211 bp, synthetic construct
  misc_feature 1..2211: note = Description of artificial sequence: Nucleic acid sequence encoding AAV9 capsid protein VP1
  source 1..2211: mol_type = other DNA
atggctgccgatggttatcttccagattggctcgaggacaaccttagtgaaggaattcgcgagtggtgggctttgaaacctggagcccctcaacccaaggcaaatcaacaacatcaagacaacgctcgaggtcttgtgcttccgggttacaaataccttggacccggcaacggactcgacaagggggagccggtcaacgcagcagacgcggcggccctcgagcacgacaaggcctacgaccagcagctcaaggccggagacaacccgtacctcaagtacaaccacgccgacgccgagttccaggagcggctcaaagaagatacgtcttttgggggcaacctcgggcgagcagtcttccaggccaaaaagaggcttcttgaacctcttggtctggttgaggaagcggctaagacggctcctggaaagaagaggcctgtagagcagtctcctcaggaaccggactcctccgcgggtattggcaaatcgggtgcacagcccgctaaaaagagactcaatttcggtcagactggcgacacagagtcagtcccagaccctcaaccaatcggagaacctcccgcagccccctcaggtgtgggatctcttacaatggcttcaggtggtggcgcaccagtggcagacaataacgaaggtgccgatggagtgggtagttcctcgggaaattggcattgcgattcccaatggctgggggacagagtcatcaccaccagcacccgaacctgggccctgcccacctacaacaatcacctctacaagcaaatctccaacagcacatctggaggatcttcaaatgacaacgcctacttcggctacagcaccccctgggggtattttgacttcaacagattccactgccacttctcaccacgtgactggcagcgactcatcaacaacaactggggattccggcctaagcgactcaacttcaagctcttcaacattcaggtcaaagaggttacggacaacaatggagtcaagaccatcgccaataaccttaccagcacggtccaggtcttcacggactcagactatcagctcccgtacgtgctcgggtcggctcacgagggctgcctcccgccgttcccagcggacgttttcatgattcctcagtacgggtatctgacgcttaatgatggaagccaggccgtgggtcgttcgtccttttactgcctggaatatttcccgtcgcaaatgctaagaacgggtaacaacttccagttcagctacgagtttgagaacgtacctttccatagcagctacgctcacagccaaagcctggaccgactaatgaatccactcatcgaccaatacttgtactatctctcaaagactattaacggttctggacagaatcaacaaacgctaaaattcagtgtggccggacccagcaacatggctgtccagggaagaaactacatacctggacccagctaccgacaacaacgtgtctcaaccactgtgactcaaaacaacaacagcgaatttgcttggcctggagcttcttcttgggctctcaatggacgtaatagcttgatgaatcctggacctgctatggccagccacaaagaaggagaggaccgtttctttcctttgtctggatctttaatttttggcaaacaaggaactggaagagacaacgtggatgcggacaaagtcatgataaccaacgaagaagaaattaaaactactaacccggtagcaacggagtcctatggacaagtggccacaaaccaccagagtgcccaagcacaggcgcagaccggctgggttcaaaaccaaggaatacttccgggtatggtttggcaggacagagatgtgtacctgcaaggacccatttgggccaaaattcctcacacggacggcaactttcacccttctccgctgatgggagggtttggaatgaagcacccgcctcctcagatcctcatcaaaaacacacctgtacctgcggatcctccaacggccttcaacaaggacaagctgaactctttcatcacccagtattctactggccaagtcagcgtggagatcgagtgggagctgcagaaggaaaacagcaagcgctggaacccggagatccagtacacttccaactattacaagtctaataatgttgaatttgctgttaatactgaaggtgtatatagtgaaccccgccccattggcaccagatacctgactcgtaatctgtaa

SEQ ID NO: 10 - protein, 736 aa, synthetic construct
  REGION 1..736: note = Description of artificial sequence: Amino acid sequence encoding AAV9 capsid protein VP1
MAADGYLPDWLEDNLSEGIREWWALKPGAPQPKANQQHQDNARGLVLPGYKYLGPGNGLDKGEPVNAADAAALEHDKAYDQQLKAGDNPYLKYNHADAEFQERLKEDTSFGGNLGRAVFQAKKRLLEPLGLVEEAAKTAPGKKRPVEQSPQEPDSSAGIGKSGAQPAKKRLNFGQTGDTESVPDPQPIGEPPAAPSGVGSLTMASGGGAPVADNNEGADGVGSSSGNWHCDSQWLGDRVITTSTRTWALPTYNNHLYKQISNSTSGGSSNDNAYFGYSTPWGYFDFNRFHCHFSPRDWQRLINNNWGFRPKRLNFKLFNIQVKEVTDNNGVKTIANNLTSTVQVFTDSDYQLPYVLGSAHEGCLPPFPADVFMIPQYGYLTLNDGSQAVGRSSFYCLEYFPSQMLRTGNNFQFSYEFENVPFHSSYAHSQSLDRLMNPLIDQYLYYLSKTINGSGQNQQTLKFSVAGPSNMAVQGRNYIPGPSYRQQRVSTTVTQNNNSEFAWPGASSWALNGRNSLMNPGPAMASHKEGEDRFFPLSGSLIFGKQGTGRDNVDADKVMITNEEEIKTTNPVATESYGQVATNHQSAQAQAQTGWVQNQGILPGMVWQDRDVYLQGPIWAKIPHTDGNFHPSPLMGGFGMKHPPPQILIKNTPVPADPPTAFNKDKLNSFITQYSTGQVSVEIEWELQKENSKRWNPEIQYTSNYYKSNNVEFAVNTEGVYSEPRPIGTRYLTRNL

SEQ ID NO: 11 - skipped

SEQ ID NO: 12 - DNA, 190 bp, synthetic construct
  misc_feature 1..190: note = Description of artificial sequence: TTR promoter Sequence
  source 1..190: mol_type = other DNA
atttcatagaacgaatgttccgatgctctaatctctctagacaaggttcatatttgtatgggttacttattctctctttgttgactaagtcaataatcagaatcagcaggtttgcagtcagattggcagggataagcagcctagctcaggagaagtgagtataaaagccccaggctgggagcagccatca

SEQ ID NO: 13 - protein, 1120 aa, synthetic construct
  REGION 1..1120: note = Description of artificial sequence: DEL 1-4 ATP7B Native, protein
MPEQERQITAREGASRKILSKLSLPTRAWEPAMKKSFAFDNVGYEGGLDGLGPSSQVATSTVRSPEELRAAIEDMGFEASVVSESCSTNPLGNHSAGNSMVQTTDGTPTSVQEVAPHTGRLPANHAPDILAKSPQSTRAVAPQKCFLQIKGMTCASCVSNIERNLQKEAGVLSVLVALMAGKAEIKYDPEVIQPLEIAQFIQDLGFEAAVMEDYAGSDGNIELTITGMTCASCVHNIESKLTRTNGITYASVALATSKALVKFDPEIIGPRDIIKIIEEIGFHASLAQRNPNAHHLDHKMEIKQWKKSFLCSLVFGIPVMALMIYMLIPSNEPHQSMVLDHNIIPGLSILNLIFFILCTFVQLLGGWYFYVQAYKSLRHRSANMDVLIVLATSIAYVYSLVILVVAVAEKAERSPVTFFDTPPMLFVFIALGRWLEHLAKSKTSEALAKLMSLQATEATVVTLGEDNLIIREEQVPMELVQRGDIVKVVPGGKFPVDGKVLEGNTMADESLITGEAMPVTKKPGSTVIAGSINAHGSVLIKATHVGNDTTLAQIVKLVEEAQMSKAPIQQLADRFSGYFVPFIIIMSTLTLVVWIVIGFIDFGVVQRYFPNPNKHISQTEVIIRFAFQTSITVLCIACPCSLGLATPTAVMVGTGVAAQNGILIKGGKPLEMAHKIKTVMFDKTGTITHGVPRVMRVLLLGDVATLPLRKVLAVVGTAEASSEHPLGVAVTKYCKEELGTETLGYCTDFQAVPGCGIGCKVSNVEGILAHSERPLSAPASHLNEAGSLPAEKDAVPQTFSVLIGNREWLRRNGLTISSDVSDAMTDHEMKGQTAILVAIDGVLCGMIAIADAVKQEAALAVHTLQSMGVDVVLITGDNRKTARAIATQVGINKVFAEVLPSHKVAKVQELQNKGKKVAMVGDGVNDSPALAQADMGVAIGTGTDVAIEAADVVLIRNDLLDVVASIHLSKRTVRRIRINLVLALIYNLVGIPIAAGVFMPIGIVLQPWMGSAAMAASSVSVVLSSLQLKCYKKPDLERYEAQAHGHMKPLTASQVSVHIGMDDRWRDSPRATPWDQVSYVSQVSLSSLTSDKPSRHSAAADDDGDKWSLLLNGRDEEQYI

SEQ ID NO: 14 - DNA, 4485 bp, synthetic construct
  misc_feature 1..4485: note = Description of artificial sequence: Expression cassette of exemplary vector DTC319
  source 1..4485: mol_type = other DNA
ttggccactccctctctgcgcgctcgctcgctcactgaggccgggcgaccaaaggtcgcccgacgcccgggctttgcccgggcggcctcagtgagcgagcgagcgcgcagagagggagtggccaactccatcactaggggttcctctacctcgtgatcgcccggcccctgttcaaacatgtcctaatactctgtctctgcaagggtcatcagtagttttccatcttactcaacatcctcccagtgatttcatagaacgaatgttccgatgctctaatctctctagacaaggttcatatttgtatgggttacttattctctctttgttgactaagtcaataatcagaatcagcaggtttgcagtcagattggcagggataagcagcctagctcaggagaagtgagtataaaagccccaggctgggagcagccatcagctctaaggtaaatataaaatttttaagtgtataatgtgttaaactactgattctaattgtttctctcttttagattccaacctttggaactgatgccgccaccatgcctgagcaggagagacagatcacagccagagaaggggccagtcggaaaatcttatctaagctttctttgcctacccgtgcctgggaaccagcaatgaagaagagttttgcttttgacaatgttggctatgaaggtggtctggatggcctgggcccttcttctcaggtggccaccagcacagtcagggatggagccgaagggagtgggacagatcacaggtcttccagttctcattcccctggctccccaccgagaaaccaggtccagggcacatgcagtaccactctgattgccattgccggcatgacctgtgcatcctgtgtccattccattgaaggcatgatctcccaactggaaggggtgcagcaaatatcggtgtctttggccgaagggactgcaacagttctttataatccctctgtaattagcccagaagaactcagagctgctatagaagacatgggatttgaggcttcagtcgtttctgaaagctgttctactaaccctcttggaaaccacagtgctgggaattccatggtgcaaactacagatggtacacctacatctgtgcaggaagtggctccccacactgggaggctccctgcaaaccatgccccggacatcttggcaaagtccccacaatcaaccagagcagtggcaccgcagaagtgcttcttacagatcaaaggcatgacctgtgcatcctgtgtgtctaacatagaaaggaatctgcagaaagaagctggtgttctctccgtgttggttgccttgatggcaggaaaggcagagatcaagtatgacccagaggtcatccagcccctcgagatagctcagttcatccaggacctgggttttgaggcagcagtcatggaggactacgcaggctccgatggcaacattgagctgacaatcacagggatgacctgcgcgtcctgtgtccacaacatagagtccaaactcacgaggacaaatggcatcacttatgcctccgttgcccttgccaccagcaaagcccttgttaagtttgacccggaaattatcggtccacgggatattatcaaaattattgaggaaattggctttcatgcttccctggcccagagaaaccccaacgctcatcacttggaccacaagatggaaataaagcagtggaagaagtctttcctgtgcagcctggtgtttggcatccctgtcatggccttaatgatctatatgctgatacccagcaacgagccccaccagtccatggtcctggaccacaacatcattccaggactgtccattctaaatctcatcttctttatcttgtgtacctttgtccagctcctcggtgggtggtacttctacgttcaggcctacaaatctctgagacacaggtcagccaacatggacgtgctcatcgtcctggccacaagcattgcttatgtttattctctggtcatcctggtggttgctgtggctgagaaggcggagaggagccctgtgacattcttcgacacgccccccatgctctttgtgttcattgccctgggccggtggctggaacacttggcaaagagcaaaacctcagaagccctggctaaactcatgtctctccaagccacagaagccaccgttgtgacccttggtgaggacaatttaatcatcagggaggagcaagtccccatggagctggtgcagcggggcgatatcgtcaaggtggtccctgggggaaagtttccagtggatgggaaagtcctggaaggcaataccatggctgatgagtccctcatcacaggagaagccatgccagtcactaagaaacccggaagcactgtaattgcggggtctataaatgcacatggctctgtgctcattaaagctacccacgtgggcaatgacaccactttggctcagattgtgaaactggtggaagaggctcagatgtcaaaggcacccattcagcagctggctgaccggtttagtggatattttgtcccatttatcatcatcatgtcaactttgacgttggtggtatggattgtaatcggttttatcgattttggtgttgttcagagatactttcctaaccccaacaagcacatctcccagacagaggtgatcatccggtttgctttccagacgtccatcacggtgctgtgcattgcctgcccctgctccctggggctggccacgcccacggctgtcatggtgggcaccggggtggccgcgcagaacggcatcctcatcaagggaggcaagcccctggagatggcgcacaagataaagactgtgatgtttgacaagactggcaccattacccatggcgtccccagggtcatgcgggtgctcctgctgggggatgtggccacactgcccctcaggaaggttctggctgtggtggggactgcggaggccagcagtgaacaccccttgggcgtggcagtcaccaaatactgtaaagaggaacttggaacagagaccttgggatactgcacggacttccaggcagtgccaggctgtggaattgggtgcaaagtcagcaacgtggaaggcatcctggcccacagtgagcgccctttgagtgcaccggccagtcacctgaatgaggctggcagccttcccgcagaaaaagatgcagtcccccagaccttctctgtgctgattggaaaccgtgagtggctgaggcgcaacggtttaaccatttctagcgatgtcagtgacgctatgacagaccacgagatgaaaggacagacagccatcctggtggctattgacggtgtgctctgtgggatgatcgcaatcgcagacgctgtcaagcaggaggctgccctggctgtgcacacgctgcagagcatgggtgtggacgtggttctgatcacgggggacaaccggaagacagccagagctattgccacccaggttggcatcaacaaagtctttgcagaggtgctgccttcgcacaaggtggccaaggtccaggagctccagaataaagggaagaaagtcgccatggtgggggatggggtcaatgactccccggccttggcccaggcagacatgggtgtggccattggcaccggcacggatgtggccatcgaggcagccgacgtcgtccttatcagaaatgatttgctggatgtggtggctagcattcacctttccaagaggactgtccgaaggatacgcatcaacctggtcctggcactgatttataacctggttgggatacccattgcagcaggtgtcttcatgcccatcggcattgtgctgcagccctggatgggctcagcggccatggcagcctcctctgtgtctgtggtgctctcatccctgcagctcaagtgctataagaagcctgacctggagaggtatgaggcacaggcgcatggccacatgaagcccctgacggcatcccaggtcagtgtgcacataggcatggatgacaggtggcgggactcccccagggccacaccatgggaccaggtcagctatgtcagccaggtgtcgctgtcctccctgacgtccgacaagccatctcggcacagcgctgcagcagacgatgatggggacaagtggtctctgctcctgaatggcagggatgaggagcagtacatctgagatccagacatgataagatacattgatgagtttggacaaaccacaactagaatgcagtgaaaaaaatgctttatttgtgaaatttgtgatgctattgctttatttgtaaccattataagctgcaataaacaagttaacaacaacaattgcattcattttatgtttcaggttcagggggaggtgtgggaggttttttagaggaacccctagtgatggagttggccactccctctctgcgcgctcgctcgctcactgaggccgcccgggcaaagcccgggcgtcgggcgacctttggtcgcccggcctcagtgagcgagcgagcgcgcagagagggagtggccaa

SEQ ID NO: 15 - DNA, 3603 bp, synthetic construct
  misc_feature 1..3603: note = Description of artificial sequence: Del 1-3 ATP7B, codon-optimized
  source 1..3603: mol_type = other DNA
atgcccgagcaggaaagacagatcaccgccagagagggcgccagccggaagatcctgagcaagctgagcctgcccaccagagcctgggagcccgccatgaagaagtccttcgccttcgacaacgtgggctacgagggcggcctggacggactgggaccatcttctcaggtggccacaagcaccgtgcgcgacggagccgagggctccggaacagatcacagaagcagcagcagccacagccctggcagcccccctagaaatcaggtgcagggcacctgtagcaccaccctgatcgccattgccggcatgacatgcgccagctgcgtgcactctattgagggcatgatctcccagctggaaggcgtgcagcagatcagtgtgtctctggccgagggcaccgccacagtgctgtacaaccctagcgtgatcagccccgaagaactgagagccgccattgaggacatgggattcgaagccagcgtggtgtccgagagctgctccaccaaccctctgggcaatcacagcgccggcaacagcatggtgcagaccaccgacggcacccccaccagcgtgcaggaagtggccccacatacaggcagactgcccgccaatcacgcccccgatatcctggccaagagcccccagagtacaagagccgtggccccccagaagtgcttcctgcagatcaagggcatgacttgtgcctcttgtgtgtccaatatcgagcggaacctgcagaaagaggccggcgtgctgtctgtgctggtggctctgatggccggcaaggccgagatcaaatacgaccccgaagtgattcagcccctggaaatcgcccagtttatccaggacctgggctttgaagccgccgtgatggaagattacgccggctccgacggcaacatcgagctgaccatcaccggaatgacctgcgcctcctgtgtgcacaacattgagtccaagctgacccggaccaacggcatcacctacgcctctgtggctctggccacctccaaggccctcgtgaagttcgatcccgagatcatcggccccagggacatcatcaagatcatcgaagagatcggcttccacgccagcctggcccagaggaaccctaacgcccaccacctggaccacaagatggaaatcaagcagtggaagaaaagcttcctgtgcagcctggtgttcggcatccccgtgatggccctgatgatctacatgctgatccccagcaacgagccccaccagtccatggtgctggatcacaacatcatccccggcctgtctatcctgaacctgatcttcttcatcctgtgcaccttcgtgcagctgctgggcggctggtacttctacgtgcaggcctacaagtccctgcggcacagatccgccaacatggacgtgctgatcgtgctggccacatctatcgcctacgtgtactccctcgtgatcctggtggtggccgtggccgagaaagccgagagaagccctgtgaccttcttcgacaccccccctatgctgttcgtgtttatcgccctgggccggtggctggaacacctggccaaaagcaagaccagcgaggccctggctaagctgatgagtctgcaggccaccgaggccacagtcgtgaccctgggcgaggacaacctgatcatccgcgaggaacaggtgccaatggaactggtgcagcggggcgacatcgtgaaggtggtgcctggcggcaagttccccgtggacggaaaagtgctggaagggaataccatggccgacgagagcctgatcacaggcgaggccatgcccgtgaccaagaaacctggcagcacagtgatcgccggcagcatcaatgcccacggcagcgtgctgattaaggccacacacgtgggcaacgataccaccctggctcagattgtgaagctggtggaagaggcccagatgagcaaggcccccattcagcagctggctgaccggttcagcggctacttcgtgccctttatcatcatcatgagcaccctgacactggtcgtgtggatcgtgatcggctttatcgacttcggagtggtgcagagatacttccccaaccctaacaagcacatcagccagacagaagtgatcatcagattcgcctttcagaccagcatcaccgtgctgtgtatcgcctgcccctgtagcctgggactggccacacctaccgctgtgatggtgggaacaggcgtggccgctcagaacggcatcctgatcaaggggggcaagcctctggaaatggctcacaagatcaagaccgtgatgttcgacaagaccggcaccatcacccacggcgtgcccagagtgatgagagtgctgctgctgggggatgtggccaccctgcctctgagaaaggtgctggctgtcgtgggcacagccgaggctagctctgaacacccactgggagtggccgtgacaaagtactgcaaagaggaactgggcaccgaaaccctgggctactgcaccgactttcaggccgtgcctggctgtggcatcggctgcaaggtgtccaacgtggaaggcatcctggcccacagcgagaggccactgtctgcccctgccagccacctgaacgaggccggatctctgcccgccgaaaaggacgctgtgccccagaccttctctgtgctgattggcaacagagagtggctgcggcggaacggcctgaccatctcctccgatgtgtccgacgccatgaccgaccacgagatgaagggccagaccgccattctggtggccattgacggggtgctgtgcggcatgatcgcaatcgccgatgccgtgaaacaggaagcagcactggccgtgcacaccctgcagtctatgggagtggatgtggtgctgatcaccggcgacaacagaaagaccgccagggccattgccacccaggtgggcatcaacaaggtgttcgccgaggtgctgcccagccacaaagtggccaaggtgcaggaactgcagaacaaaggcaaaaaggtggccatggtgggagatggcgtgaacgactctcctgctctggcccaggcagatatgggcgtggccatcggcacaggcaccgacgtggcaattgaggctgctgacgtggtgctgattcggaacgacctgctggacgtggtggcctccatccacctgtccaagagaaccgtgcggcggatcagaatcaacctggtgctggcactgatctataacctcgtgggcatccctatcgccgctggcgtgttcatgcctatcggaatcgtgctgcagccctggatgggctctgccgccatggctgcaagctccgtgtctgtggtgctgtccagcctgcagctgaagtgctacaagaagcccgacctggaaagatacgaggcccaggcccacggacacatgaagcctctgacagcctcccaggtgtccgtgcacatcggcatggacgacagatggcgggacagccctagagccaccccttgggatcaggtgtcatacgtgtcacaggtgtccctgagcagcctgaccagcgacaagcccagcagacatagcgccgctgccgacgacgatggggacaagtggtccctgctgctgaacggccgggatgaggaacagtacatctga